European Patent Application EP 4 628 593 A1, published October 8, 2025. Title: Method for Detecting Methylation and Mutation States of DNA Sample. Applicant: NANODIGMBIO (NANJING) BIOTECHNOLOGY CO., LTD. The sequence listing filed with the application follows.

SEQUENCE LISTING (219 sequences)

SEQ ID NO: 1 - DNA, 52 bp, synthetic construct
  source 1..52: mol_type = other DNA; note = 5' biotin
cgtcggtcgggagagcggtgggaagtattcgcctccgttcctcacaccgacg

SEQ ID NO: 2 - DNA, 50 bp, synthetic construct
  source 1..50: mol_type = other DNA; note = 5' biotin
cgtcggtcgacaggatgcgagcgccctttggagaagtcgcgccaccgacg

SEQ ID NO: 3 - DNA, 51 bp, synthetic construct
  source 1..51: mol_type = other DNA; note = 5' biotin
cgtcggtcggcggaaacgctaactccccggccaagtgcaaatgcaccgacg

SEQ ID NO: 4 - DNA, 52 bp, synthetic construct
  source 1..52: mol_type = other DNA; note = 5' biotin
cgtcggtcggcacacacgagggcccgtcgcgccccccgccctgccaccgacg

SEQ ID NO: 5 - DNA, 51 bp, synthetic construct
  source 1..51: mol_type = other DNA; note = 5' biotin
cgtcggtcggcctcgccctccacgtccctgcacccccaagtcgcaccgacg

SEQ ID NO: 6 - DNA, 51 bp, synthetic construct
  source 1..51: mol_type = other DNA; note = 5' biotin
cgtcggtcgtaagaacccagtccccgatcggtttcctctacgccaccgacg

SEQ ID NO: 7 - DNA, 51 bp, synthetic construct
  source 1..51: mol_type = other DNA; note = 5' biotin
cgtcggtcgggagggagggggggaaagggggacgaggggcggacaccgacg

SEQ ID NO: 8 - DNA, 52 bp, synthetic construct
  source 1..52: mol_type = other DNA; note = 5' biotin
cgtcggtcgggggggtttggaagcgcactgccacttgcaaagtccaccgacg

SEQ ID NO: 9 - DNA, 52 bp, synthetic construct
  source 1..52: mol_type = other DNA; note = 5' biotin
cgtcggtcgacccgagcaatcacagccggagcgcgattcgaatgcaccgacg

SEQ ID NO: 10 - DNA, 51 bp, synthetic construct
  source 1..51: mol_type = other DNA; note = 5' biotin
cgtcggtcgtgaaccgaagacctcgtaggcgggcctcggggggcaccgacg

SEQ ID NO: 11 - DNA, 52 bp, synthetic construct
  source 1..52: mol_type = other DNA; note = 5' biotin
cgtcggtcggatgccgttggcggcggccagcgccagcccctcggcaccgacg

SEQ ID NO: 12 - DNA, 51 bp, synthetic construct
  source 1..51: mol_type = other DNA; note = 5' biotin
cgtcggtcggtgccgtagagcagctgcagctcgcgcgcctcgtcaccgacg

SEQ ID NO: 13 - DNA, 51 bp, synthetic construct
  source 1..51: mol_type = other DNA; note = 5' biotin
cgtcggtcgggctcaggtcgccgcagcccgggagcctccccgccaccgacg

SEQ ID NO: 14 - DNA, 51 bp, synthetic construct
  source 1..51: mol_type = other DNA; note = 5' biotin
cgtcggtcggccccaaggcacgcgcggcacagccatgaacacccaccgacg

SEQ ID NO: 15 - DNA, 51 bp, synthetic construct
  source 1..51: mol_type = other DNA; note = 5' biotin
cgtcggtcggatgccaaggagtatctggcccggagggaaatcccaccgacg

SEQ ID NO: 16 - DNA, 51 bp, synthetic construct
  source 1..51: mol_type = other DNA; note = 5' biotin
cgtcggtcggagtcccgcgcgctctccgtgcgccccggccggccaccgacg

SEQ ID NO: 17 - DNA, 52 bp, synthetic construct
  source 1..52: mol_type = other DNA; note = 5' biotin
cgtcggtcggcggcggctgccgcgcacaggcttccgactccagccaccgacg

SEQ ID NO: 18 - DNA, 51 bp, synthetic construct
  source 1..51: mol_type = other DNA; note = 5' biotin
cgtcggtcgcggcccgccactgagcatgcccagcacgccggcccaccgacg

SEQ ID NO: 19 - DNA, 52 bp, synthetic construct
  source 1..52: mol_type = other DNA; note = 5' biotin
cgtcggtcggagcggaggggacagcggggatcgtgagctccggccaccgacg

SEQ ID NO: 20 - DNA, 52 bp, synthetic construct
  source 1..52: mol_type = other DNA; note = 5' biotin
cgtcggtcggggcgagcgggtgcgtctgccgcagagtcggcacccaccgacg

SEQ ID NO: 21 - DNA, 52 bp, synthetic construct
  source 1..52: mol_type = other DNA; note = 5' biotin
cgtcggtcgaaggacatggaggtaaaggaccccggagggagacgcaccgacg

SEQ ID NO: 22 - DNA, 52 bp, synthetic construct
  source 1..52: mol_type = other DNA; note = 5' biotin
cgtcggtcggcacgtgcggcgctcagcttaggctctcggaggcacaccgacg

SEQ ID NO: 23 - DNA, 52 bp, synthetic construct
  source 1..52: mol_type = other DNA; note = 5' biotin
cgtcggtcgtgagttggaaatcccgacggaaagcacccacaagccaccgacg

SEQ ID NO: 24 - DNA, 51 bp, synthetic construct
  source 1..51: mol_type = other DNA; note = 5' biotin
cgtcggtcgcactctgcgctggcccacccgcgtgcacgcccaccaccgacg

SEQ ID NO: 25 - DNA, 51 bp, synthetic construct
  source 1..51: mol_type = other DNA; note = 5' biotin
cgtcggtcggcggagctaagcaggggtgtttggaaggcgcccgcaccgacg

SEQ ID NO: 26 - DNA, 50 bp, synthetic construct
  source 1..50: mol_type = other DNA; note = 5' biotin
cgtcggtcggctgtttgactgcgtggcttcacttggcccgcgcaccgacg

SEQ ID NO: 27 - DNA, 52 bp, synthetic construct
  source 1..52: mol_type = other DNA; note = 5' biotin
cgtcggtcgatcagcctctctggcgggggattctccccggactccaccgacg

SEQ ID NO: 28 - DNA, 52 bp, synthetic construct
  source 1..52: mol_type = other DNA; note = 5' biotin
cgtcggtcgggcgggcggggagccaggcccgagctgcgttctgccaccgacg

SEQ ID NO: 29 - DNA, 51 bp, synthetic construct
  source 1..51: mol_type = other DNA; note = 5' biotin
cgtcggtcgagccattggtgggcgccgcgctctgcactgagcacaccgacg

SEQ ID NO: 30 - DNA, 52 bp, synthetic construct
  source 1..52: mol_type = other DNA; note = 5' biotin
cgtcggtcgtcgcgccccgccggcccctagccgcagccgcagcccaccgacg

SEQ ID NO: 31 - DNA, 52 bp, synthetic construct
  source 1..52: mol_type = other DNA; note = 5' biotin
cgtcggtcgggcaggcggcaggacggggatcccaggctgcggggcaccgacg

SEQ ID NO: 32 - DNA, 52 bp, synthetic construct
  source 1..52: mol_type = other DNA; note = 5' biotin
cgtcggtcgactccgcggcagagccgctgggacctgacccgggacaccgacg

SEQ ID NO: 33 - DNA, 52 bp, synthetic construct
  source 1..52: mol_type = other DNA; note = 5' biotin
cgtcggtcggccttcgtccccgcgcgcacctccccgggtcgggccaccgacg

SEQ ID NO: 34 - DNA, 50 bp, synthetic construct
  source 1..50: mol_type = other DNA; note = 5' biotin
cgtcggtcgaaggggggctggtggaatctggcggtccccagccaccgacg

SEQ ID NO: 35 - DNA, 51 bp, synthetic construct
  source 1..51: mol_type = other DNA; note = 5' biotin
cgtcggtcgcgtgtcccgggtcggtgcgctcggcgcacccgtgcaccgacg

SEQ ID NO: 36 - DNA, 52 bp, synthetic construct
  source 1..52: mol_type = other DNA; note = 5' biotin
cgtcggtcggacagtgcccggcgtctgctcccacccgcccgccccaccgacg

SEQ ID NO: 37 - DNA, 52 bp, synthetic construct
  source 1..52: mol_type = other DNA; note = 5' biotin
cgtcggtcggaacttgccggtggtggggtcgtagtggtttccgacaccgacg

SEQ ID NO: 38 - DNA, 52 bp, synthetic construct
  source 1..52: mol_type = other DNA; note = 5' biotin
cgtcggtcgttggtgaccacgtcgtcgaacttgagcacctcgtacaccgacg

SEQ ID NO: 39 - DNA, 51 bp, synthetic construct
  source 1..51: mol_type = other DNA; note = 5' biotin
cgtcggtcgttcatgctgccgcttgaggccggcgtagaaggcgcaccgacg

SEQ ID NO: 40 - DNA, 51 bp, synthetic construct
  source 1..51: mol_type = other DNA; note = 5' biotin
cgtcggtcgggcggcccgggcaccgcgagccggccgagctccacaccgacg

SEQ ID NO: 41 - DNA, 51 bp, synthetic construct
  source 1..51: mol_type = other DNA; note = 5' biotin
cgtcggtcgggagctacgtgactacgtccacccgcacctacagcaccgacg

SEQ ID NO: 42 - DNA, 52 bp, synthetic construct
  source 1..52: mol_type = other DNA; note = 5' biotin
cgtcggtcgtgggcagcgcgctgcgccccagcaccagccgcagccaccgacg

SEQ ID NO: 43 - DNA, 52 bp, synthetic construct
  source 1..52: mol_type = other DNA; note = 5' biotin
cgtcggtcgggcgccgggcccgcgatcggagccggaggcaccgccaccgacg

SEQ ID NO: 44 - DNA, 52 bp, synthetic construct
  source 1..52: mol_type = other DNA; note = 5' biotin
cgtcggtcgagcggaaagagggctccgcggcggccaggctcagccaccgacg

SEQ ID NO: 45 - DNA, 52 bp, synthetic construct
  source 1..52: mol_type = other DNA; note = 5' biotin
cgtcggtcgtgccgggaaaatgctggatttaactcccagtctgccaccgacg

SEQ ID NO: 46 - DNA, 51 bp, synthetic construct
  source 1..51: mol_type = other DNA; note = 5' biotin
cgtcggtcgtcccggggatgccagactcctggggacgctgggacaccgacg

SEQ ID NO: 47 - DNA, 50 bp, synthetic construct
  source 1..50: mol_type = other DNA; note = 5' biotin
cgtcggtcggcggcgcggcgggacacgcaggactcccgcctccaccgacg

SEQ ID NO: 48 - DNA, 52 bp, synthetic construct
  source 1..52: mol_type = other DNA; note = 5' biotin
cgtcggtcggcccggaattcgttgagacggaatctcagcggatccaccgacg

SEQ ID NO: 49 - DNA, 51 bp, synthetic construct
  source 1..51: mol_type = other DNA; note = 5' biotin
cgtcggtcgtggggagaagcgctgcggaaaggggcgactccgacaccgacg

SEQ ID NO: 50 - DNA, 52 bp, synthetic construct
  source 1..52: mol_type = other DNA; note = 5' biotin
cgtcggtcgagatggccctgtcccggcgccccaggtcgtcgcgccaccgacg

SEQ ID NO: 51 - DNA, 52 bp, synthetic construct
  source 1..52: mol_type = other DNA; note = 5' biotin
cgtcggtcggcagctgcggtagtcactgcgcctccccgcccccacaccgacg

SEQ ID NO: 52 - DNA, 51 bp, synthetic construct
  source 1..51: mol_type = other DNA; note = 5' biotin
cgtcggtcgctggatgccccccttccctctcccggccagactccaccgacg

SEQ ID NO: 53 - DNA, 50 bp, synthetic construct
  source 1..50: mol_type = other DNA; note = 5' biotin
cgtcggtcgcggtgctgtgtgcctggccggagcgttttgaaacaccgacg

SEQ ID NO: 54 - DNA, 52 bp, synthetic construct
  source 1..52: mol_type = other DNA; note = 5' biotin
cgtcggtcgtccggggccgctcggcggcgctgcgattggccgcgcaccgacg

SEQ ID NO: 55 - DNA, 50 bp, synthetic construct
  source 1..50: mol_type = other DNA; note = 5' biotin
cgtcggtcggggtaacctctatgcaaatgaggccgcgccgcccaccgacg

SEQ ID NO: 56 - DNA, 51 bp, synthetic construct
  source 1..51: mol_type = other DNA; note = 5' biotin
cgtcggtcggcgggctcggcccggtccctccgctggggggttacaccgacg

SEQ ID NO: 57 - DNA, 51 bp, synthetic construct
  source 1..51: mol_type = other DNA; note = 5' biotin
cgtcggtcgagccggccggcagcgagatacccagaggcccgttcaccgacg

SEQ ID NO: 58 - DNA, 51 bp, synthetic construct
  source 1..51: mol_type = other DNA; note = 5' biotin
cgtcggtcgcaccgcgttgccatagcaacggcctggccggctgcaccgacg

SEQ ID NO: 59 - DNA, 52 bp, synthetic construct
  source 1..52: mol_type = other DNA; note = 5' biotin
cgtcggtcggaggtgccggctgcacaacggcgcccacgtgaccccaccgacg

SEQ ID NO: 60 - DNA, 51 bp, synthetic construct
  source 1..51: mol_type = other DNA; note = 5' biotin
cgtcggtcggtgcagccccaggcgcgcccaagggcagctcgcccaccgacg

SEQ ID NO: 61 - DNA, 52 bp, synthetic construct
  source 1..52: mol_type = other DNA; note = 5' biotin
cgtcggtcggagaaggacctaaaaccccgtctggggcacagaggcaccgacg

SEQ ID NO: 62 - DNA, 52 bp, synthetic construct
  source 1..52: mol_type = other DNA; note = 5' biotin
cgtcggtcgacatctggggaaaccgaggcgcagagcgggacggccaccgacg

SEQ ID NO: 63 - DNA, 52 bp, synthetic construct
  source 1..52: mol_type = other DNA; note = 5' biotin
cgtcggtcgtgggcctggcgggaagtcgcgcaaggaggccggcacaccgacg

SEQ ID NO: 64 - DNA, 52 bp, synthetic construct
  source 1..52: mol_type = other DNA; note = 5' biotin
cgtcggtcggggcgcacccggcccaccctgtcccttccaggccgcaccgacg

SEQ ID NO: 65 - DNA, 52 bp, synthetic construct
  source 1..52: mol_type = other DNA; note = 5' biotin
cgtcggtcggctgcagcacaggctgcagggggcgggcagcgccgcaccgacg

SEQ ID NO: 66 - DNA, 51 bp, synthetic construct
  source 1..51: mol_type = other DNA; note = 5' biotin
cgtcggtcgtctagcggggcaggcgagcggagcagcagcgttccaccgacg

SEQ ID NO: 67 - DNA, 52 bp, synthetic construct
  source 1..52: mol_type = other DNA; note = 5' biotin
cgtcggtcgagccccggccgcggcccctgagaggcgcgcactcgcaccgacg

SEQ ID NO: 68 - DNA, 52 bp, synthetic construct
  source 1..52: mol_type = other DNA; note = 5' biotin
cgtcggtcggcctccctgtgccagccggctgtcgacccaggttacaccgacg

SEQ ID NO: 69 - DNA, 52 bp, synthetic construct
  source 1..52: mol_type = other DNA; note = 5' biotin
cgtcggtcgaagcccgaggtcggggcgttaccccaagggccctccaccgacg

SEQ ID NO: 70 - DNA, 52 bp, synthetic construct
  source 1..52: mol_type = other DNA; note = 5' biotin
cgtcggtcggcttcccctccgagggcagagaggcgtccgcgccccaccgacg

SEQ ID NO: 71 - DNA, 52 bp, synthetic construct
  source 1..52: mol_type = other DNA; note = 5' biotin
cgtcggtcgggggctgcggggtccgtggaacctttccgggaggccaccgacg

SEQ ID NO: 72 - DNA, 52 bp, synthetic construct
  source 1..52: mol_type = other DNA; note = 5' biotin
cgtcggtcggccgcgggctgctgggcgcggaggctggagccgcgcaccgacg

SEQ ID NO: 73 - DNA, 52 bp, synthetic construct
  source 1..52: mol_type = other DNA; note = 5' biotin
cgtcggtcgaggttcggctgctgaagcggccactgcctcccagacaccgacg

SEQ ID NO: 74 - DNA, 52 bp, synthetic construct
  source 1..52: mol_type = other DNA; note = 5' biotin
cgtcggtcggatcgatggagagaaggcgggcaagacgccgggaacaccgacg

SEQ ID NO: 75 - DNA, 52 bp, synthetic construct
  source 1..52: mol_type = other DNA; note = 5' biotin
cgtcggtcggcattcctcctcaaccgagtgccacaaccgccctccaccgacg

SEQ ID NO: 76 - DNA, 51 bp, synthetic construct
  source 1..51: mol_type = other DNA; note = 5' biotin
cgtcggtcggaagtgccccggggcttcgagcatcacctcgcggcaccgacg

SEQ ID NO: 77 - DNA, 52 bp, synthetic construct
  source 1..52: mol_type = other DNA; note = 5' biotin
cgtcggtcgagctgagaccggcggccgacggccagccctcagggcaccgacg

SEQ ID NO: 78 - DNA, 51 bp, synthetic construct
  source 1..51: mol_type = other DNA; note = 5' biotin
cgtcggtcgggtcacaagtcagcgcccaagcaagtcaagcgaccaccgacg

SEQ ID NO: 79 - DNA, 51 bp, synthetic construct
  source 1..51: mol_type = other DNA; note = 5' biotin
cgtcggtcggctcgtcttcgcccgaactgatgcgctgcaaacgcaccgacg

SEQ ID NO: 80 - DNA, 52 bp, synthetic construct
  source 1..52: mol_type = other DNA; note = 5' biotin
cgtcggtcgggctcaacttcagcggctttggctacagcctgccgcaccgacg

SEQ ID NO: 81 - DNA, 51 bp, synthetic construct
  source 1..51: mol_type = other DNA; note = 5' biotin
cgtcggtcggagcgcaaccgcgtcaagttggtcaacctgggctcaccgacg

SEQ ID NO: 82 - DNA, 51 bp, synthetic construct
  source 1..51: mol_type = other DNA; note = 5' biotin
cgtcggtcgcacccttcgggagcacgtccccaacggcgcggcccaccgacg

SEQ ID NO: 83 - DNA, 51 bp, synthetic construct
  source 1..51: mol_type = other DNA; note = 5' biotin
cgtcggtcgaagaagatgagtaaggtggagacactgcgctcggcaccgacg

SEQ ID NO: 84 - DNA, 50 bp, synthetic construct
  source 1..50: mol_type = other DNA; note = 5' biotin
cgtcggtcgtggccctggttgggtccgcccgcagcgagggcgcaccgacg

SEQ ID NO: 85 - DNA, 52 bp, synthetic construct
  source 1..52: mol_type = other DNA; note = 5' biotin
cgtcggtcgagacctgcgaagaagttcggaaacttttccagtggcaccgacg

SEQ ID NO: 86 - DNA, 52 bp, synthetic construct
  source 1..52: mol_type = other DNA; note = 5' biotin
cgtcggtcggctgctgggagctgtcagggggctgccggattcgccaccgacg

SEQ ID NO: 87 - DNA, 52 bp, synthetic construct
  source 1..52: mol_type = other DNA; note = 5' biotin
cgtcggtcggccgaggctgggagcgcggtgatggccggtccccgcaccgacg

SEQ ID NO: 88 - DNA, 52 bp, synthetic construct
  source 1..52: mol_type = other DNA; note = 5' biotin
cgtcggtcgagcagagggcagcggcggcgggaccggggactctgcaccgacg

SEQ ID NO: 89 - DNA, 51 bp, synthetic construct
  source 1..51: mol_type = other DNA; note = 5' biotin
cgtcggtcgcaatgggtaaagccaggaggaagcccgtgcctggcaccgacg

SEQ ID NO: 90 - DNA, 52 bp, synthetic construct
  source 1..52: mol_type = other DNA; note = 5' biotin
cgtcggtcgaggcgggcaggaggggaggagtagggaggcgagagcaccgacg

SEQ ID NO: 91 - DNA, 52 bp, synthetic construct
  source 1..52: mol_type = other DNA; note = 5' biotin
cgtcggtcggcgggcgggaggcgccacggcctctcagacgctggcaccgacg

SEQ ID NO: 92 - DNA, 51 bp, synthetic construct
  source 1..51: mol_type = other DNA; note = 5' biotin
cgtcggtcgccgcagccgagaagccagagagaaagttcccgggcaccgacg

SEQ ID NO: 93 - DNA, 51 bp, synthetic construct
  source 1..51: mol_type = other DNA; note = 5' biotin
cgtcggtcggcagtaagcgagtaagcgagccctggagaccgggcaccgacg

SEQ ID NO: 94 - DNA, 51 bp, synthetic construct
  source 1..51: mol_type = other DNA; note = 5' biotin
cgtcggtcgctgggtgtgcggtcggctcagtgccacgcggtgacaccgacg

SEQ ID NO: 95 - DNA, 51 bp, synthetic construct
  source 1..51: mol_type = other DNA; note = 5' biotin
cgtcggtcgtaggcatggttatcaacccacgccaaggcggttgcaccgacg

SEQ ID NO: 96 - DNA, 52 bp, synthetic construct
  source 1..52: mol_type = other DNA; note = 5' biotin
cgtcggtcggctgcctcgccccggagcccggaggaggggagccgcaccgacg

SEQ ID NO: 97 - DNA, 51 bp, synthetic construct
  source 1..51: mol_type = other DNA; note = 5' biotin
cgtcggtcgacccggggaagaagcggaggacgccgatctggcccaccgacg

SEQ ID NO: 98 - DNA, 51 bp, synthetic construct
  source 1..51: mol_type = other DNA; note = 5' biotin
cgtcggtcgtgcgttgcgcgctccaaccctctgcttggccgcccaccgacg

SEQ ID NO: 99 - DNA, 52 bp, synthetic construct
  source 1..52: mol_type = other DNA; note = 5' biotin
cgtcggtcgacaaatccccgaggcggggagactttcagggcatccaccgacg

SEQ ID NO: 100 - DNA, 52 bp, synthetic construct
  source 1..52: mol_type = other DNA; note = 5' biotin
cgtcggtcggatgctgaagcctcgcggtccccattcccaagccccaccgacg

SEQ ID NO: 101 - DNA, 51 bp, synthetic construct
  source 1..51: mol_type = other DNA; note = 5' biotin
cgtcggtcgccgtgcgccgcctgcgcgtggcgcagttaatttgcaccgacg

SEQ ID NO: 102 - DNA, 51 bp, synthetic construct
  source 1..51: mol_type = other DNA; note = 5' biotin
cgtcggtcggtcttgaggtggggaggggagaaatgggaagaggcaccgacg

SEQ ID NO: 103 - DNA, 51 bp, synthetic construct
  source 1..51: mol_type = other DNA; note = 5' biotin
cgtcggtcgagtagcggttttagcccgctctgcggctgcgaggcaccgacg

SEQ ID NO: 104 - DNA, 52 bp, synthetic construct
  source 1..52: mol_type = other DNA; note = 5' biotin
cgtcggtcgagatccgagattaacctctcccgcgataggtgaagcaccgacg

SEQ ID NO: 105 - DNA, 51 bp, synthetic construct
  source 1..51: mol_type = other DNA; note = 5' biotin
cgtcggtcgttggggcgacggggccaggcgcgggggacggctgcaccgacg

SEQ ID NO: 106 - DNA, 52 bp, synthetic construct
  source 1..52: mol_type = other DNA; note = 5' biotin
cgtcggtcgggctgggagggcgcgcggaggagacaccgctgaggcaccgacg

SEQ ID NO: 107 - DNA, 52 bp, synthetic construct
  source 1..52: mol_type = other DNA; note = 5' biotin
cgtcggtcgacgccgctgagggcgccacgcggggggcgcggctgcaccgacg

SEQ ID NO: 108 - DNA, 52 bp, synthetic construct
  source 1..52: mol_type = other DNA; note = 5' biotin
cgtcggtcgagtgcgcacttgaggcgcgggacgcaccggctgtgcaccgacg

SEQ ID NO: 109 - DNA, 52 bp, synthetic construct
  source 1..52: mol_type = other DNA; note = 5' biotin
cgtcggtcgtcccaggggctgagactcgcgccccgccccgcagccaccgacg

SEQ ID NO: 110 - DNA, 52 bp, synthetic construct
  source 1..52: mol_type = other DNA; note = 5' biotin
cgtcggtcgtcggctcgccgggccgggcccctctccggaacctccaccgacg

SEQ ID NO: 111 - DNA, 52 bp, synthetic construct
  source 1..52: mol_type = other DNA; note = 5' biotin
cgtcggtcggcggctggaggacgcgctgctgcggatgcgcgaggcaccgacg

SEQ ID NO: 112 - DNA, 52 bp, synthetic construct
  source 1..52: mol_type = other DNA; note = 5' biotin
cgtcggtcgtacgggatacaggccgaggagcggcaggtccgtgccaccgacg

SEQ ID NO: 113 - DNA, 52 bp, synthetic construct
  source 1..52: mol_type = other DNA; note = 5' biotin
cgtcggtcgggggatggcgcgctgaccccatacccgctgccgtccaccgacg

SEQ ID NO: 114 - DNA, 51 bp, synthetic construct
  source 1..51: mol_type = other DNA; note = 5' biotin
cgtcggtcgcggctgcggggccgccgccgagcgagggcgaggacaccgacg

SEQ ID NO: 115 - DNA, 52 bp, synthetic construct
  source 1..52: mol_type = other DNA; note = 5' biotin
cgtcggtcggcaccgtgcgcttcgcccgcaaaggcgccctccggcaccgacg

SEQ ID NO: 116 - DNA, 52 bp, synthetic construct
  source 1..52: mol_type = other DNA; note = 5' biotin
cgtcggtcggaagaacgtgcatgaggtcaagaaccacaaattcacaccgacg

SEQ ID NO: 117 - DNA, 51 bp, synthetic construct
  source 1..51: mol_type = other DNA; note = 5' biotin
cgtcggtcggatggccgcgccgccccgggggagccggagccgacaccgacg

SEQ ID NO: 118 - DNA, 52 bp, synthetic construct
  source 1..52: mol_type = other DNA; note = 5' biotin
cgtcggtcgtggccgccgcccgcgcgcactcaccaagcccgctgcaccgacg

SEQ ID NO: 119 - DNA, 51 bp, synthetic construct
  source 1..51: mol_type = other DNA; note = 5' biotin
cgtcggtcgtcctcctcgcacgagtaccagatgccggtgtggacaccgacg

SEQ ID NO: 120 - DNA, 52 bp, synthetic construct
  source 1..52: mol_type = other DNA; note = 5' biotin
cgtcggtcgtccctgggccgggactggagcgcaaacggttgggacaccgacg

SEQ ID NO: 121 - DNA, 51 bp, synthetic construct
  source 1..51: mol_type = other DNA; note = 5' biotin
cgtcggtcgtgtcggtgtctgcccgcccgtctgtgcgtctgtccaccgacg

SEQ ID NO: 122 - DNA, 52 bp, synthetic construct
  source 1..52: mol_type = other DNA; note = 5' biotin
cgtcggtcgtgtcggtgtgagcgtctgaggcgatggggaagacacaccgacg

SEQ ID NO: 123 - DNA, 51 bp, synthetic construct
  source 1..51: mol_type = other DNA; note = 5' biotin
cgtcggtcggggcgcttctagtcggacaaaatgcagccgagaacaccgacg

SEQ ID NO: 124 - DNA, 51 bp, synthetic construct
  source 1..51: mol_type = other DNA; note = 5' biotin
cgtcggtcgcgctcgttctgtgcgttctcctgtcccaggtaggcaccgacg

SEQ ID NO: 125 - DNA, 52 bp, synthetic construct
  source 1..52: mol_type = other DNA; note = 5' biotin
cgtcggtcgagaggggctgccgggcgcgctctgcgccccgtttccaccgacg

SEQ ID NO: 126 - DNA, 51 bp, synthetic construct
  source 1..51: mol_type = other DNA; note = 5' biotin
cgtcggtcgtgggagcagggtgtccgaagcgcgggtaccgatccaccgacg

SEQ ID NO: 127 - DNA, 52 bp, synthetic construct
  source 1..52: mol_type = other DNA; note = 5' biotin
cgtcggtcgggcagcgcggggcacgcggcgcgcgggcgagtctgcaccgacg

SEQ ID NO: 128 - DNA, 51 bp, synthetic construct
  source 1..51: mol_type = other DNA; note = 5' biotin
cgtcggtcgtgcgcgcgcggacgccttggttcccggagcccagcaccgacg

SEQ ID NO: 129 - DNA, 51 bp, synthetic construct
  source 1..51: mol_type = other DNA; note = 5' biotin
cgtcggtcgccaccttctcagtccgggacgcgagacgggaacgcaccgacg

SEQ ID NO: 130 - DNA, 51 bp, synthetic construct
  source 1..51: mol_type = other DNA; note = 5' biotin
cgtcggtcggccctggcgccccaacgctgcaccaccgtgggtccaccgacg

SEQ ID NO: 131 - DNA, 52 bp, synthetic construct
  source 1..52: mol_type = other DNA; note = 5' biotin
cgtcggtcggagccgtgctcgcagtcgctgagatcctcggtgcgcaccgacg

SEQ ID NO: 132 - DNA, 52 bp, synthetic construct
  source 1..52: mol_type = other DNA; note = 5' biotin
cgtcggtcggcgtctctcgccgtcccctgggcgcgggccaggcgcaccgacg

SEQ ID NO: 133 - DNA, 51 bp, synthetic construct
  source 1..51: mol_type = other DNA; note = 5' biotin
cgtcggtcggaggaggggggcgctccggtcgtgtgcccaggaccaccgacg

SEQ ID NO: 134 - DNA, 51 bp, synthetic construct
  source 1..51: mol_type = other DNA; note = 5' biotin
cgtcggtcgccccagcggccactcgggccccagccccccaggccaccgacg

SEQ ID NO: 135 - DNA, 52 bp, synthetic construct
  source 1..52: mol_type = other DNA; note = 5' biotin
cgtcggtcgtggagatttagagcccgggaatgaggcgccgtgtccaccgacg

SEQ ID NO: 136 - DNA, 52 bp, synthetic construct
  source 1..52: mol_type = other DNA; note = 5' biotin
cgtcggtcgtaggaatctcgcgcccggggagcgctgagggaccgcaccgacg

SEQ ID NO: 137 - DNA, 52 bp, synthetic construct
  source 1..52: mol_type = other DNA; note = 5' biotin
cgtcggtcggagccgggtggggagcgggcctcggggcgcccggccaccgacg

SEQ ID NO: 138 - DNA, 52 bp, synthetic construct
  source 1..52: mol_type = other DNA; note = 5' biotin
cgtcggtcggcagggccggaaggaggcccctgccccgtccaaggcaccgacg

SEQ ID NO: 139 - DNA, 52 bp, synthetic construct
  source 1..52: mol_type = other DNA; note = 5' biotin
cgtcggtcggcaccagctgccccgccgcccgcccggacccagcccaccgacg

SEQ ID NO: 140 - DNA, 52 bp, synthetic construct
  source 1..52: mol_type = other DNA; note = 5' biotin
cgtcggtcggcctcattgctgacgagaccccgccctgctactcccaccgacg

SEQ ID NO: 141 - DNA, 52 bp, synthetic construct
  source 1..52: mol_type = other DNA; note = 5' biotin
cgtcggtcgggccggagaaggcgccgctggggccgcccggaggacaccgacg

SEQ ID NO: 142 - DNA, 50 bp, synthetic construct
  source 1..50: mol_type = other DNA; note = 5' biotin
cgtcggtcgcctctgcacgggcccgtggagacgcttcctgcgcaccgacg

SEQ ID NO: 143 - DNA, 52 bp, synthetic construct
  source 1..52: mol_type = other DNA; note = 5' biotin
cgtcggtcgaaccttctggaatccaccgcccccctttccgcccgcaccgacg

SEQ ID NO: 144 - DNA, 51 bp, synthetic construct
  source 1..51: mol_type = other DNA; note = 5' biotin
cgtcggtcgcgcgcccgcccccaggagggcctccgcgagccggcaccgacg

SEQ ID NO: 145 - DNA, 52 bp, synthetic construct
  source 1..52: mol_type = other DNA; note = 5' biotin
cgtcggtcggcacaccccgaggcggtcccggctgcacaacttggcaccgacg

SEQ ID NO: 146 - DNA, 51 bp, synthetic construct
  source 1..51: mol_type = other DNA; note = 5' biotin
cgtcggtcggagttgctccgtttcctcattttgggggcgaagacaccgacg

SEQ ID NO: 147 - DNA, 52 bp, synthetic construct
  source 1..52: mol_type = other DNA; note = 5' biotin
cgtcggtcggccggcggcggccagtagcggcgccgtgtgcagggcaccgacg

SEQ ID NO: 148 - DNA, 52 bp, synthetic construct
  source 1..52: mol_type = other DNA; note = 5' biotin
cgtcggtcgagcgccgcctgcgccgcgttcagcacgaagagctccaccgacg

SEQ ID NO: 149 - DNA, 52 bp, synthetic construct
  source 1..52: mol_type = other DNA; note = 5' biotin
cgtcggtcgtccagctcaggcgcagcagcgccacctggtcggcccaccgacg

SEQ ID NO: 150 - DNA, 52 bp, synthetic construct
  source 1..52: mol_type = other DNA; note = 5' biotin
cgtcggtcgggcgcccgcattggtgctgacataatttcctgacccaccgacg

SEQ ID NO: 151 - DNA, 53 bp, synthetic construct
  source 1..53: mol_type = other DNA; note = 5' biotin
cgtcggtcgtgacccgtattgtctcgcgattaaaggtaaaaaacgcaccgacg

SEQ ID NO: 152 - DNA, 52 bp, synthetic construct
  source 1..52: mol_type = other DNA; note = 5' biotin
cgtcggtcggctttttcatcccactggggtaaaacgcccttttacaccgacg

SEQ ID NO: 153 - DNA, 52 bp, synthetic construct
  source 1..52: mol_type = other DNA; note = 5' biotin
cgtcggtcgagtggggccgcggggcctgctgggaggtgttgtcccaccgacg

SEQ ID NO: 154 - DNA, 52 bp, synthetic construct
  source 1..52: mol_type = other DNA; note = 5' biotin
cgtcggtcgggaaacgtcgctggcgcggagggatggttcggcgccaccgacg

SEQ ID NO: 155 - DNA, 51 bp, synthetic construct
  source 1..51: mol_type = other DNA; note = 5' biotin
cgtcggtcgtaggcgtctgtcacagacctatctgcgggtcgcccaccgacg

SEQ ID NO: 156 - DNA, 50 bp, synthetic construct
  source 1..50: mol_type = other DNA; note = 5' biotin
cgtcggtcgccagcgccatagcccttaggactatcggtcacacaccgacg

SEQ ID NO: 157 - DNA, 50 bp, synthetic construct
  source 1..50: mol_type = other DNA; note = 5' biotin
cgtcggtcctcgcgctcctgctccggctcctccatcttggcccaccgacg

SEQ ID NO: 158 - DNA, 50 bp, synthetic construct
  source 1..50: mol_type = other DNA; note = 5' biotin
cgtcggtcggagcagagcgaggtgtgtgcctccttaccgcctcaccgacg

SEQ ID NO: 159 - DNA, 51 bp, synthetic construct
  source 1..51: mol_type = other DNA; note = 5' biotin
cgtcggtcgtgcactggacgtccttccccagcagccagttgagcaccgacg

SEQ ID NO: 160 - DNA, 51 bp, synthetic construct
  source 1..51: mol_type = other DNA; note = 5' biotin
cgtcggtcagacggaggctggtggtgcagcaggcaggcaagaccaccgacg

SEQ ID NO: 161 - DNA, 51 bp, synthetic construct
  source 1..51: mol_type = other DNA; note = 5' biotin
cgtcggtcgatgccggggactacagctgcgaggccaggggccacaccgacg

SEQ ID NO: 162 - DNA, 51 bp, synthetic construct
  source 1..51: mol_type = other DNA; note = 5' biotin
cgtcggtcgcacagcgttgtgcatccaggtctagcgtgtcttccaccgacg

SEQ ID NO: 163 - DNA, 55 bp, synthetic construct
  source 1..55: mol_type = other DNA; note = 5' biotin
cgtcggtcctgtcttctgtggatgaggtatatgaatttatcccaaagcaccgacg

SEQ ID NO: 164 - DNA, 51 bp, synthetic construct
  source 1..51: mol_type = other DNA; note = 5' biotin
cgtcggtccgagacctcccagagcccgtggttccctggagccacaccgacg

SEQ ID NO: 165 - DNA, 51 bp, synthetic construct
  source 1..51: mol_type = other DNA; note = 5' biotin
cgtcggtctacgaagggttcctgctctgtgggcagctcacgaacaccgacg

SEQ ID NO: 166 - DNA, 56 bp, synthetic construct
  source 1..56: mol_type = other DNA; note = 5' biotin
cgtcggtccaataatgcacatggagaaagttcacctacaataaagaggcaccgacg

SEQ ID NO: 167 - DNA, 55 bp, synthetic construct
  source 1..55: mol_type = other DNA; note = 5' biotin
cgtcggtctgtattggtaacattttatatcgaattcctgttctatgtcaccgacg

SEQ ID NO: 168 - DNA, 51 bp, synthetic construct
  source 1..51: mol_type = other DNA; note = 5' biotin
cgtcggtcagatgtcccctccctgtccgtccccgcacctggagcaccgacg

SEQ ID NO: 169 - DNA, 51 bp, synthetic construct
  source 1..51: mol_type = other DNA; note = 5' biotin
cgtcggtctggtggtgcatgcccgaacccagcacttccttgaacaccgacg

SEQ ID NO: 170 - DNA, 50 bp, synthetic construct
  source 1..50: mol_type = other DNA; note = 5' biotin
cgtcggtccaactggccaacctagagcccccctggtaaaagccaccgacg

SEQ ID NO: 171 - DNA, 55 bp, synthetic construct
  source 1..55: mol_type = other DNA; note = 5' biotin
cgtcggtctcttggtggaatagatgttaattagtttttttattactccaccgacg

SEQ ID NO: 172 - DNA, 51 bp, synthetic construct
  source 1..51: mol_type = other DNA; note = 5' biotin
cgtcggtcggaaacaattctgtgttcaccctcaccctgcaggccaccgacg

SEQ ID NO: 173 - DNA, 51 bp, synthetic construct
  source 1..51: mol_type = other DNA; note = 5' biotin
cgtcggtcggcctctcagccatcaagacaccgtatcctacctccaccgacg

SEQ ID NO: 174 - DNA, 51 bp, synthetic construct
  source 1..51: mol_type = other DNA; note = 5' biotin
cgtcggtcacgtgctgagcgcacgcacgtggcgcctgctcacccaccgacg

SEQ ID NO: 175 - DNA, 51 bp, synthetic construct
  source 1..51: mol_type = other DNA; note = 5' biotin
cgtcggtcgatgctgctccagcgcccgcgcgagttgcggatcgcaccgacg

SEQ ID NO: 176 - DNA, 56 bp, synthetic construct
  source 1..56: mol_type = other DNA; note = 5' biotin
cgtcggtcgtagttgacaaatacatttagtgatgtcttacttttttggcaccgacg

SEQ ID NO: 177 - DNA, 51 bp, synthetic construct
  source 1..51: mol_type = other DNA; note = 5' biotin
cgtcggtcatctcctaccagtgtatccttcacgacagacgcaccaccgacg

SEQ ID NO: 178 - DNA, 51 bp, synthetic construct
  source 1..51: mol_type = other DNA; note = 5' biotin
cgtcggtccgagcgatgatgacaccaaatccatgtgtccaccccaccgacg

SEQ ID NO: 179 - DNA, 50 bp, synthetic construct
  source 1..50: mol_type = other DNA; note = 5' biotin
cgtcggtcgggacccaggagggcacagccaaggaatgagccccaccgacg

SEQ ID NO: 180 - DNA, 51 bp, synthetic construct
  source 1..51: mol_type = other DNA; note = 5' biotin
cgtcggtcctcctggtcagcagcctcttagagaacctgctggacaccgacg

SEQ ID NO: 181 - DNA, 52 bp, synthetic construct
  source 1..52: mol_type = other DNA; note = 5' biotin
cgtcggtctatagaaccatcatcatgcaagatgagagcaaggagcaccgacg

SEQ ID NO: 182 - DNA, 56 bp, synthetic construct
  source 1..56: mol_type = other DNA; note = 5' biotin
cgtcggtcgaacagtaaacagtggttctgactggtgaaatgatagttacaccgacg

SEQ ID NO: 183 - DNA, 55 bp, synthetic construct
  source 1..55: mol_type = other DNA; note = 5' biotin
cgtcggtcgttgaaaggaccagcactttatttattgctttagccattcaccgacg

SEQ ID NO: 184 - DNA, 51 bp, synthetic construct
  source 1..51: mol_type = other DNA; note = 5' biotin
cgtcggtcagcctgcacgggagtcagaggcactcagcaatgcccaccgacg

SEQ ID NO: 185 - DNA, 50 bp, synthetic construct
  source 1..50: mol_type = other DNA; note = 5' biotin
cgtcggtctggctctgttacgaacggctgaaatcaaaacccccaccgacg

SEQ ID NO: 186 - DNA, 51 bp, synthetic construct
  source 1..51: mol_type = other DNA; note = 5' biotin
cgtcggtctcaccgtgttctccagaccatgcatgttcctccgccaccgacg

SEQ ID NO: 187 - DNA, 51 bp, synthetic construct
  source 1..51: mol_type = other DNA; note = 5' biotin
cgtcggtcaccgccccttcagggatggggctgtaggagtcaagcaccgacg

SEQ ID NO: 188 - DNA, 51 bp, synthetic construct
  source 1..51: mol_type = other DNA; note = 5' biotin
cgtcggtctctcggtgtctccccaggtgcaagtgcaacctgcacaccgacg

SEQ ID NO: 189 - DNA, 51 bp, synthetic construct
  source 1..51: mol_type = other DNA; note = 5' biotin
cgtcggtcgccaacctgtgctccatgcgcgagggcagcctgcacaccgacg

SEQ ID NO: 190 - DNA, 51 bp, synthetic construct
  source 1..51: mol_type = other DNA; note = 5' biotin
cgtcggtcaagcccactcttctactccccgaacgtgccttccccaccgacg

SEQ ID NO: 191 - DNA, 51 bp, synthetic construct
  source 1..51: mol_type = other DNA; note = 5' biotin
cgtcggtcctctgacggcgacagtagctccgtggacagcgatgcaccgacg

SEQ ID NO: 192 - DNA, 51 bp, synthetic construct
  source 1..51: mol_type = other DNA; note = 5' biotin
cgtcggtcctggaggagcacggaaaagacctggaaatcatgcacaccgacg

SEQ ID NO: 193 - DNA, 51 bp, synthetic construct
  source 1..51: mol_type = other DNA; note = 5' biotin
cgtcggtcatcctcaccagggtgaatgacagagttgccaggcacaccgacg

SEQ ID NO: 194 - DNA, 51 bp, synthetic construct
  source 1..51: mol_type = other DNA; note = 5' biotin
cgtcggtcgcataggagtaggccagccagcggaacacgtggtccaccgacg

SEQ ID NO: 195 - DNA, 51 bp, synthetic construct
  source 1..51: mol_type = other DNA; note = 5' biotin
cgtcggtctcgggggtgggggtgtgttcctgcgtcttccagggcaccgacg

SEQ ID NO: 196 - DNA, 51 bp, synthetic construct
  source 1..51: mol_type = other DNA; note = 5' biotin
cgtcggtccgggaatgccgagtaagtgttaattttatggtccccaccgacg

SEQ ID NO: 197 - DNA, 56 bp, synthetic construct
  source 1..56: mol_type = other DNA; note = 5' biotin
cgtcggtcatcacttctggaaaatgaatagatagatgtgtgggctttacaccgacg

SEQ ID NO: 198 - DNA, 54 bp, synthetic construct
  source 1..54: mol_type = other DNA; note = 5' biotin
cgtcggtcgtgcctcaatgatcttttttccccaccttcatttttctcaccgacg

SEQ ID NO: 199 - DNA, 50 bp, synthetic construct
  source 1..50: mol_type = other DNA; note = 5' biotin
cgtcggtccttcagcggcatctgctagctcgtctacccctgtcaccgacg

SEQ ID NO: 200 - DNA, 54 bp, synthetic construct
  source 1..54: mol_type = other DNA; note = 5' biotin
cgtcggtccatgttttagggaactctgccctataaacactcatagacaccgacg

SEQ ID NO: 201 - DNA, 51 bp, synthetic construct
  source 1..51: mol_type = other DNA; note = 5' biotin
cgtcggtcggtttctctctatgttgcagtccctctgtcgtgaacaccgacg

SEQ ID NO: 202 - DNA, 50 bp, synthetic construct
  source 1..50: mol_type = other DNA; note = 5' biotin
cgtcggtccggcattcctgtggtagtggcctgagaacacgaccaccgacg

SEQ ID NO: 203 - DNA, 51 bp, synthetic construct
  source 1..51: mol_type = other DNA; note = 5' biotin
cgtcggtctgacacctgcagagaagggaaaaagtcattaggggcaccgacg

SEQ ID NO: 204 - DNA, 51 bp, synthetic construct
  source 1..51: mol_type = other DNA; note = 5' biotin
cgtcggtcacatgtccctgcgtcacaggcacctgcagagcccccaccgacg

SEQ ID NO: 205 - DNA, 51 bp, synthetic construct
  source 1..51: mol_type = other DNA; note = 5' biotin
cgtcggtctgtgtaaggcgttccggcacgtcaaggtggacacacaccgacg

SEQ ID NO: 206 - DNA, 51 bp, synthetic construct
  source 1..51: mol_type = other DNA; note = 5' biotin
cgtcggtctgaagatacaaacaaccacagcagcctgcacttaccaccgacg

SEQ ID NO: 207 - DNA, 51 bp, synthetic construct
  source 1..51: mol_type = other DNA; note = 5' biotin
cgtcggtcgtgtggtcatcttcttcttccccttctagcacgaccaccgacg

SEQ ID NO: 208 - DNA, 51 bp, synthetic construct
  source 1..51: mol_type = other DNA; note = 5' biotin
cgtcggtcacgttgcatcgaccctctccactccgcggaagtagcaccgacg

SEQ ID NO: 209 - DNA, 50 bp, synthetic construct
  source 1..50: mol_type = other DNA; note = 5' biotin
cgtcggtccgacaccgtctgatgtgttgcgcaggtggtggcacaccgacg

SEQ ID NO: 210 - DNA, 51 bp, synthetic construct
  source 1..51: mol_type = other DNA; note = 5' biotin
cgtcggtccattgggatggagggtggggaaggagtcaccctggcaccgacg

SEQ ID NO: 211 - DNA, 50 bp, synthetic construct
  source 1..50: mol_type = other DNA; note = 5' biotin
cgtcggtccctcctccgcctgacttacttgatcctaaagtcacaccgacg

SEQ ID NO: 212 - DNA, 50 bp, synthetic construct
  source 1..50: mol_type = other DNA; note = 5' biotin
cgtcggtcctcccagggctccttggcctcctccgcggtgacccaccgacg

SEQ ID NO: 213 - DNA, 51 bp, synthetic construct
  source 1..51: mol_type = other DNA; note = 5' biotin
cgtcggtcgggacacagggccgcatgagcctgggcggggtcagcaccgacg

SEQ ID NO: 214 - DNA, 51 bp, synthetic construct
  source 1..51: mol_type = other DNA; note = 5' biotin
cgtcggtccgccctccgaggagggcccgggcggggtgggcgcccaccgacg

SEQ ID NO: 215 - DNA, 50 bp, synthetic construct
  source 1..50: mol_type = other DNA; note = 5' biotin
cgtcggtccgtcctcaggctccaggctgggaggagagagcgtcaccgacg

SEQ ID NO: 216 - DNA, 51 bp, synthetic construct
  source 1..51: mol_type = other DNA; note = 5' biotin
cgtcggtcgctgggagtggagctgggggtcagaagagcaagcacaccgacg

SEQ ID NO: 217 - DNA, 54 bp, synthetic construct
  source 1..54: mol_type = other DNA; note = 5' biotin
cgtcggtcaacgaaattgatcaaacttagactgcttcacctgtctccaccgacg

SEQ ID NO: 218 - DNA, 51 bp, synthetic construct
  source 1..51: mol_type = other DNA; note = 5' biotin
cgtcggtcgcgtggacaggcagcgccgcagtgacgtctccatgcaccgacg

SEQ ID NO: 219 - DNA, 51 bp, synthetic construct
  source 1..51: mol_type = other DNA; note = 5' biotin
cgtcggtctggagtcctccagcggcttcaggcggttcagcttccaccgacg